European Patent Specification EP 4 003 412 B1, published June 24, 2026. Title: Vaccine. Applicant: The Pirbright Institute. The sequence listing filed with the application follows.

SEQUENCE LISTING (19 sequences)

SEQ ID NO: 1 - protein, 674 aa, Artificial Sequence
  African swine fever virus (ASFV) polypeptide, B602L (OUR T88/3)
MAEFNIDELLKNVLEDPSTEISEETLKQLYQRTNPYKQFKNDSRVAFCSFTNLREQYIRRLIMTSFIGYVFKALQEWMPSYSKPTHTTKTLLSELITLVDTLKQETNDVPSESVVNTILSIADSCKTQTQKSKEAKTTIDSFLREHFVFDPNLHAQSAYTCASTCADTNVDTCASTCASTCASTCASTCASTCASTCASTCASTCASTCASTCASTCASTCASTGASTGASTCADTNVDTCASTCADTNVDTCASTCASTCASTCASTCASTGASTCADTNVDTCASTCADTNVDTCASTCADTNVDTCASTCADTNVNTCASMCADTNVDTCASTCANTCASTEYTDLADPERIPLHIMQKTLNVPNELQADIDAITQTPQGYRAAAHILQNIELHQSIKHMLENPRAFKPILFNTKITRYLSQHIPPQDTFYKWNYYIEDNYEELRAATESIYPEKPDLEFAFIIYDVVDSSNQQKVDEFYYKYKDQIFSEVSSIQLGNWTLLGSFKANRERYNYFNQNNEIIKRILDRHEEDLKIGKEILRNTIYHKKAKNIQETGPDAPGLSIYNSTFHTDSGIKGLLSFKELKNLEKASGNIKKAREYDFIDDCEEKIKQLLSKENLTPDEESELIKTKKQLNNALEMLNVPDDTIRVDMWVNNNNKLEKEILYTKAEL

SEQ ID NO: 2 - protein, 183 aa, Artificial Sequence
  ASFV polypeptide, E183L (p54) (OUR T88/3)
MDSEFFQPVYPRHYGECLSPVTPPSFFSTHMYTILIAIVVLVIIIIVLIYLFSSRKKKAAAAIEEEDIQFINPYQDQQWAEVTPQPGTSKPAGATTASAGKPVTGRPATNRPATNKPVTDNPVTDRLVMATGGPAAAPAAASAHPTEPYTTVTTQNTASQTMSAIENLRQRNTYTHKDLENSL

SEQ ID NO: 3 - protein, 153 aa, Artificial Sequence
  ASFV polypeptide, EP153R (Benin 1997/1)
MYFKKKYIGLIDKNCEKKILDDSSTIKICYILIGILIGTNMITLIYNFIFWDNYIKCYRNNDKMFYCPNDWVGYNNICYYFSNGSFSKNYTAASNFCRQLNGTLANNDTNLLNLTKIYNNQSMYWVNNTVILRGDNKYSQKVNYTDLLFICGK

SEQ ID NO: 4 - protein, 646 aa, Artificial Sequence
  ASFV polypeptide, B646L (OUR T88/3)
MASGGAFCLIANDGKADKIILAQDLLNSRISNIKNVNKSYGKPDPEPTLSQIEETHLVHFNAHFKPYVPVGFEYNKVRPHTGTPTLGNKLTFGIPQYGDFFHDMVGHHILGACHSSWQDAPIQGTAQMGAHGQLQTFPRNGYDWDNQTPLEGAVYTLVDPFGRPIVPGTKNAYRNLVYYCEYPGERLYENVRFDVNGNSLDEYSSDVTTLVRKFCIPGDKMTGYKHLVGQEVSVEGTSGPLLCNIHDLHKPHQSKPILTDENDTQRTCSHTNPKFLSQHFPENSHNIQTAGKQDITPITDATYLDIRRNVHYSCNGPQTPKYYQPPLALWIKLRFWFNENVNLAIPSVSIPFGERFITIKLASQKDLVNEFPGLFIRQSRFIPGRPSRRNIRFKPWFIPGVINEISLTNNELYINNLFVTPEIHNLFVKRVRFSLIRVHKTQVTHTNNNHHDEKLMSALKWPIEYMFIGLKPTWNISDQNPHQHRDWHKFGHVVNAIMQPTHHAEISFQDRDTALPDACSSISDISPVTYPITLPIIKNISVTAHGINLIDKFPSKFCSSYIPFHYGGNAIKTPDDPGAMMITFALKPREEYQPSGHINVSRAREFYISWDTDYVGSITTADLVVSASAINFLLLQNGSAVLRYST

SEQ ID NO: 5 - protein, 194 aa, Artificial Sequence
  ASFV polypeptide, CP204L (p30) (OUR T88/3)
MDFILNISMKMEVIFKTDLRSSSQVVFHAGSLYNWFSVEIINSGRIVTTAIKTLLSTVKYDIVKSAHIYAGQGYTEHQAQEEWNMILHVLFEEETESSASSESIHEKNDNETNECASSFETLFEQEPSSEEPKDSKLYMLAQKTVQHIEQYGKAPDFNKVIRAHNFIQTIHGTPLKEEEKEVVRLMVIKLLKKK

SEQ ID NO: 6 - protein, 199 aa, Artificial Sequence
  ASFV polypeptide, E199L (OUR T88/3)
MSCMPVSTKCNDIWVDFSCTGPSISELQKKEPKAWAAILRSHTNQQTAEDDNIIGSICDKRGLCSKDEYAYSQYCACVNSGTLWAECAFAPCNGNKNAYKTTEQRNILTNKQCPSGLTICQNIAEYRGSGNISDLYQNFNCNSVINTFLINVMNHPFLTLILIILILIIIYRLMPSSGGKHNDDKLPPPSLIFSNLNNF

SEQ ID NO: 7 - protein, 317 aa, Artificial Sequence
  ASFV polypeptide, F317L (OUR T88/3)
MVETQMDKLGFLLNHIGKQVTTKVLSNAHITQTMKEIILENHGVDGGAAKNVSKGKSSPKEKKHWTEFESWEQLSKSKRSFKEYWAERNEIVNTLLLNWDNVRGAIKKFLDDDREWCGRINMINGVPEIVEIIPSPYRAGENIYFGSEAMMPADIYSRVANKPAMFVFHTHPNLGSCCGGMPSICDISTTLRYLLMGWTAGHLIISSNQVGMLTVDKRIIVDLWANENPRWLMAQKILDIFMMLTSRRSLVNPWTLRDLKKILQDYGIEYIIFPSNDFFIYEDERLLMFSKKWTNFFTLHELLDDLETIETKASSTT

SEQ ID NO: 8 - protein, 498 aa, Artificial Sequence
  ASFV polypeptide, MGF505-5R (OUR T88/3)
MFSLQEICRKNIYFLPDWLSEHVIQRLGLYWEKHGSLQRIGDDYVLIQQDLIIPINEALRMAGEEGNDEVVQLLLLWEGNIHYAIIGALESDHYSLIRKLYDQIGDCHDILPLIQDPKIFEKCHELDKFCNILCLVLHAVKNDMLCILQEYKMHLSGEDIQVVFETACRSQKNDIVSWMGQNIAIYNSGVIFDIAFDKMNVSLLSIGYTLLFNHHINNTNENINSLLTQHLEWAAGMGLLHFMLETLKYGGDVTIIVLSEAVKYDHRKILDYFLRRKNLYQEDLEELLLLAIRADCSKKTLNLLLSYLNYSINNIRKKILQCVKEYETTVIIKILWKRKINLIEPILADFIGYHSYTYMVDFMREFSIHPEKMIKMAARESREDLIIKFSKKVCKEPKDRLHYLKSLVYTMRHKEGKQLLIYTIHNLYKACHLESKEMFNLARFYARHNAVIQFKSICHDLSKLNINIKNLLLECLGIAIKKNYFQLIKTIETDMRYE

SEQ ID NO: 9 - DNA, 2025 bp, Artificial Sequence
  nucleic acid sequence encoding ASFV polypeptide B602L (OUR T88/3)
atggcagaatttaatattgatgagcttctcaaaaacgtattggaggatccctctactgaaatatccgaagaaacgcttaaacagctttatcaaaggacgaacccttacaaacagttcaaaaatgatagcagggtggccttttgctcttttacaaatttgcgggagcagtatattcgacgtcttataatgactagctttattggatatgtcttcaaagctctgcaggaatggatgccttcctattcaaaacctacccacacgaccaaaactcttctcagtgagctaataacgttagttgatactttgaaacaggaaactaatgatgttccctctgaatcggtagtaaatacaattttatctatagcggatagctgcaaaacccagacgcagaaaagcaaggaagctaaaacaacgatcgatagctttttacgagaacattttgtgtttgatcctaatcttcatgctcaaagtgcgtatacttgtgcaagcacttgtgcagataccaatgtagacacctgtgcaagcacttgtgcaagcacttgtgcaagcacttgtgcaagcacttgtgcaagcacttgtgcaagcacttgtgcaagcacttgtgcaagcacttgtgcaagcacttgtgcaagcacttgtgcaagcacttgtgcaagcacttgtgcaagcacaggtgcaagcacaggtgcaagcacttgtgcagataccaatgtagacacctgtgcaagcacttgtgcagataccaatgtagacacctgtgcaagcacttgtgcaagcacttgtgcaagcacttgtgcaagcacttgtgcaagcacaggtgcaagcacttgtgcagataccaatgtagacacctgtgcaagcacttgtgcagataccaatgtagacacctgtgcaagcacttgtgcagataccaatgtagacacctgtgcaagcacttgtgcagataccaatgtaaacacttgtgcaagcatgtgtgcagataccaatgtagacacctgtgcaagcacctgtgcaaacacctgtgcaagcacagaatacaccgatttagcagatcctgagcgcatccctttacacatcatgcaaaaaacattaaatgtgcctaatgagcttcaggccgatattgatgcaattacccaaaccccacagggctatagggcagcagcccacatattacaaaatatagaacttcatcaaagcattaaacatatgcttgaaaatccgagggcgtttaaacccattctctttaacacaaaaattactagatatctttcgcagcatattccacctcaggatactttttataagtggaattattacattgaggataattacgaagagttgcgggccgctacggaaagcatctacccagaaaagcccgacctagagtttgccttcattatttatgatgtggtggatagcagcaaccaacaaaaggttgatgaattttattataaatataaagaccagattttctcagaggtttcatccattcaattaggcaactggacactcctgggaagctttaaggccaacagagagcgctacaattattttaatcaaaataatgaaataataaaacggattttggaccgtcatgaggaagacctaaagataggaaaagagattctacgaaataccatttaccacaaaaaagcaaaaaatatacaagaaaccggcccggatgctccggggctctccatctataattcaacctttcacacggatagcgggattaagggactgctttcctttaaggagctaaaaaacctagaaaaagcatctggaaatatcaaaaaagctcgagagtatgattttatagacgactgcgaagaaaaaattaagcaactgcttagtaaagaaaatttaacccccgatgaagaaagcgagctgataaaaacaaaaaaacagttaaataatgcgcttgaaatgctcaatgtgcctgatgatacgatacgggtagatatgtgggtcaacaataataataaactcgaaaaagaaattttatatacaaaagcagaattgtaa

SEQ ID NO: 10 - DNA, 552 bp, Artificial Sequence
  nucleic acid sequence encoding E183L (p54) (OUR T88/3)
atggattctgaattttttcaaccggtttatccgcggcattatggtgagtgtttgtcaccagtcaccccaccaagcttcttctccacacatatgtatactattctcattgctatcgtggtcttagtcattattatcatcgttctaatctatctattctcttcaagaaagaaaaaagctgctgccgctattgaggaggaagatatacagtttataaatccttatcaagatcagcaatgggcagaagtcactccacaaccaggtacctctaaaccggctggagcgactacagcaagtgcaggcaaaccagtcacgggcagaccggcaacaaacagaccagcaacaaacaaaccagtcacggacaacccagttacggacagactagtcatggcaactggcgggccagcggccgcacctgcggccgcgagtgctcatccgactgagccttacacgacagtcactactcagaacactgcttcacaaacaatgtcggctattgaaaatttacgacaaagaaacacctatacgcataaagacctagaaaactccttgtaa

SEQ ID NO: 11 - DNA, 462 bp, Artificial Sequence
  nucleic acid sequence encoding EP153R (Benin 1997/1)
atgtattttaagaaaaaatacatcggtcttattgataagaactgtgaaaaaaaaatattagatgattctagtacaataaaaatttgttacatattaattggaatattgattggaactaatatgataactcttatttataatttcatattctgggataattatataaaatgttaccgaaataatgataaaatgttttactgtcctaatgattgggttggatataataatatttgttactattttagtaatggtagtttttctaaaaattatacagctgctagtaatttttgtagacaattaaatggtacacttgctaataatgatactaatttattaaatctaactaaaatatataataatcaatctatgtattgggttaacaatacggtaatattacgtggtgataataaatatagtcaaaaagttaactatacagatttattatttatttgtggtaaataa

SEQ ID NO: 12 - DNA, 1941 bp, Artificial Sequence
  nucleic acid sequence encoding B646L (OUR T88/3)
atggcatcaggaggagctttttgtcttattgctaacgatgggaaggccgacaagattatattggcccaagacttgcttaatagcaggatttctaacattaaaaatgtgaacaaaagttatgggaaacccgaccccgaacccactttgagtcaaatcgaagaaacacatttggttcattttaatgcgcattttaagccttatgttccagtagggtttgaatacaataaagtacgcccgcatacgggtacccccaccttgggaaacaagcttacctttggtattccccagtacggagactttttccatgatatggtgggccaccatatattgggtgcatgtcattcgtcctggcaggatgctccgattcagggcacggcccagatgggggcccatggtcagcttcaaacgtttcctcgcaacggatatgactgggacaaccaaacacctttagagggcgccgtttacacgcttgtagatccctttggaagacctattgtacccggcacaaagaatgcgtaccgaaacttggtttactactgcgaataccccggagaacgactttatgaaaacgtaagattcgatgtaaatggaaattccctggacgaatatagttcggatgtcacaacgcttgtgcgcaaattttgcatcccaggggataaaatgactggatataagcacttggtcggccaggaggtatcggtggagggaactagtggccctctcctatgcaacattcatgatttgcacaagccgcaccaaagcaaacctattcttaccgatgaaaatgatacgcagcgaacgtgcagccataccaacccgaaattcctttcacaacattttcccgagaactctcacaatatccaaacagcaggtaaacaagatattactcctattacggacgcaacgtatctggacataagacgtaatgttcattacagctgtaatggacctcaaacccctaaatactatcagccccctcttgcgctctggattaagctgcgcttttggtttaacgagaacgtgaaccttgctattccctcggtatccattcccttcggcgagcgctttatcaccataaagcttgcatcgcaaaaggatttggtgaatgaatttcctggactttttatacgccagtcgcgttttatacctggacgccccagtagacgcaatatacgctttaaaccatggtttatcccaggagtcattaatgaaatctcgctcacgaataatgaactttacatcaataacctgtttgtaacccctgaaatacacaacctttttgtaaaacgcgttcgattttccctgatacgtgtccataaaacgcaggtgacccacaccaacaataaccaccacgatgaaaaactaatgtctgctcttaaatggcccattgaatatatgtttataggattaaaacctacctggaacatctccgatcaaaatcctcatcaacaccgagattggcacaagttcggacatgttgttaacgccattatgcagcctactcaccacgcagagataagctttcaggatagagatacagctcttccagacgcatgttcatctatatcggatattagccccgttacgtatccgatcacattacctattattaaaaacatttccgtaactgctcatggtatcaatcttatcgataagtttccatcaaagttctgcagctcttacatacccttccactacggaggcaatgcaattaaaacccccgatgatccgggtgcgatgatgattacctttgctttgaagccacgggaggaataccaacccagtggtcatattaacgtatccagagcaagagaattttatattagttgggacacggattacgtggggtctatcactacggctgatcttgtggtatcggcatctgctattaactttcttcttcttcagaacggttcagctgtgctgcgttacagtacctaa

SEQ ID NO: 13 - DNA, 585 bp, Artificial Sequence
  nucleic acid sequence encoding CP204L (p30) (OUR T88/3)
atggattttattttaaatatatccatgaaaatggaggtcatcttcaaaacggatttaagatcatcttcacaagttgtgtttcatgcgggtagcttgtataattggttttctgttgagattatcaatagcggtagaattgttacgaccgctataaaaacattgctcagtactgttaagtatgatattgtgaaatctgctcatatatatgcagggcaagggtatactgaacatcaggctcaagaagaatggaatatgattctgcatgtgctgtttgaagaggagacagaatcctcagcatcatcggaaagcattcatgaaaaaaatgataatgaaaccaatgaatgcgcatcctcctttgaaacattgtttgagcaagagccctcatcagaggaacctaaagactccaagctgtatatgcttgcacaaaagactgtgcaacatattgaacaatatggaaaggcacctgattttaacaaggttattagagcacataactttattcaaaccattcatggaacccctctaaaggaagaagaaaaagaggtggtaagactcatggtcattaaacttttaaaaaaaaaataa

SEQ ID NO: 14 - DNA, 600 bp, Artificial Sequence
  nucleic acid sequence encoding E199L (OUR T88/3)
atgtcttgcatgccagtttccacgaaatgcaatgatatttgggtcgactttagctgtacaggcccttcgatttccgagctgcaaaaaaaggagcccaaggcctgggccgctattttacgctcgcatacaaatcaacaaacggcggaggatgacaatattattgggagcatatgcgataaacggggattgtgctcaaaggatgagtatgcgtatagccagtattgtgcctgtgtgaactccggcaccctatgggctgaatgtgcgtttgctccgtgtaatggaaataaaaatgcctataaaacaacggagcaaagaaatattttgaccaacaagcagtgcccctccggactcaccatatgtcagaacattgcagaatacagaggctcgggcaatatttccgacctataccaaaatttcaactgcaacagcgttataaatacgtttttaattaatgtgatgaatcatccttttttaacccttatattaatcattttgattcttataattatttaccgtttgatgccttccagtgggggtaaacacaatgacgataagttgccccctccatctcttattttttcaaacctaaacaatttttaa

SEQ ID NO: 15 - DNA, 954 bp, Artificial Sequence
  nucleic acid sequence encoding F317L (OUR T88/3)
atggttgagacacaaatggacaaacttggttttctgctaaatcacataggtaaacaggttaccactaaggtgcttagcaatgcccatataactcaaacgatgaaggagattattttggaaaatcatggtgtagatggtggagccgcaaaaaatgtttcaaaagggaagtcttccccaaaagaaaaaaaacattggaccgagttcgaatcctgggaacagctcagcaagtctaaaagaagtttcaaggaatactgggcggagcgtaatgagattgtgaacactctgttgcttaattgggacaatgttcggggtgccatcaaaaaatttttggacgatgaccgtgaatggtgcggccgcattaatatgataaacggtgtacccgagatagtggaaatcattccaagcccctatagggcaggagagaacatttattttggcagcgaggctatgatgcctgctgatatttatagcagggtggccaacaagcctgctatgtttgtgtttcacacgcatcctaatttgggttcatgttgtggaggaatgccttccatatgtgacatttctacaacgctgcgttatctacttatggggtggaccgccgggcatctaatcatttcttcgaatcaagtaggaatgctcacggttgataagagaattattgttgatttgtgggccaatgagaatccgcgctggctcatggcgcaaaaaatattagatatttttatgatgctcacttcgcgtagaagcctggtaaatccctggaccctgagagacctaaaaaaaatattacaagactatggtattgagtatatcatttttccttcgaatgacttttttatttatgaagacgaacgtcttttaatgttttcaaaaaaatggaccaacttttttacgttacatgagttattggatgacctcgaaactattgagacaaaggcatcgtccacaacatag

SEQ ID NO: 16 - DNA, 1497 bp, Artificial Sequence
  nucleic acid sequence encoding MGF505-5R (OUR T88/3)
atgttctccctccaggagatctgtcgaaagaacatctactttctacctgactggctcagtgagcatgtgattcagcgactaggtctgtactgggaaaaacatggttctcttcagcgaatcggagacgactatgtacttatacaacaggatctcatcatccccatcaatgaagctctaagaatggcaggggaggaggggaatgatgaggtggtacaactcctattactatgggagggaaacattcattatgccatcataggagctttggagagtgaccattatagcctaatacgtaagctctatgaccaaatcggagactgtcacgacatccttcccttaattcaagacccaaaaatctttgaaaaatgccatgaattagataaattttgtaacattttatgtctcgtattacacgccgtaaaaaacgatatgctttgcattcttcaagagtataaaatgcatctaagtggagaggatattcaagtggtgtttgaaacagcatgccgttcacaaaaaaacgatattgtgtcatggatgggacaaaatattgcaatatacaactccggagttatttttgatattgcctttgataagatgaatgtgtccttattatctatagggtacacgcttcttttcaatcatcatataaataatacgaacgaaaatattaattctttattgacacaacatcttgaatgggctgccggcatgggccttcttcattttatgctggaaactttaaagtatggcggggatgtaacgataatagttttgtctgaggccgtaaaatatgaccacagaaagattttagattattttctccgtcgaaaaaacttgtaccaagaagatcttgaagaactattattgttggcgatacgtgcagattgttctaaaaagaccttaaacttgttattatcttacttaaactattccataaacaatatccgtaaaaaaatattacaatgtgtaaaagaatatgaaacgaccgttattataaaaattctatggaaaagaaagataaatctgatagagcccattttggcagactttataggatatcatagctatacctatatggtagattttatgcgcgagttttccatccatccggaaaaaatgatcaaaatggctgcgcgagaatcgagggaggacttaatcataaaattttccaaaaaagtttgcaaagagcctaaagatagacttcactatctcaaaagcttagtgtatactatgcgacataaagaaggcaaacaactgttaatttatacaatccataacttatacaaagcttgtcatctagagagtaaagaaatgtttaatttggcacgattttatgcacggcataatgcagtgatccagttcaaatcgatttgtcacgatctctccaagctgaatattaatatcaaaaacttgttgttagaatgtttaggtattgctattaaaaaaaattactttcaacttatcaaaacaatagaaacggatatgcgttatgagtaa

SEQ ID NO: 17 - protein, 158 aa, Artificial Sequence
  ASFV polypeptide, 17 EP153R (Genotype II)
MFSNKKYIGLINKKEGLKKKIDDYSILIIGILIGTNILSLIINIIGEINKPICYQNDDKIFYCPKDWVGYNNVCYYFGNEEKNYNNASNYCKQLNSTLTNNNTILVNLTKTLNLTKTYNHESNYWVNYSLIKNESVLLRDSGYYKKQKHVSLLYICSK

SEQ ID NO: 18 - protein, 20 aa, Foot-and-mouth disease virus
QCTNYALLKLAGDVESNPGP

SEQ ID NO: 19 - protein, 20 aa, Foot-and-mouth disease virus
RAEGRGSLLTCGDVEENPGP